European Patent Specification EP 3 735 981 B1, published August 30, 2023. Title: MOTILE SPERM DOMAIN CONTAINING PROTEIN 2 AND INFLAMMATION. Applicant: VASCULAR BIOGENICS LTD. The sequence listing filed with the application follows.

SEQUENCE LISTING (15 sequences)

SEQ ID NO: 1 - protein, 518 aa, Homo sapiens
  motile sperm domain containing 2, protein variant 1
MAENHAQNKAKLISETRRRFEAEYVTDKSDKYDARDVERLQQDDNWVESYLSWRHNIVDETLKMLDESFQWRKEISVNDLNESSIPRWLLEIGVIYLHGYDKEGNKLFWIRVKYHVKDQKTILDKKKLIAFWLERYAKRENGKPVTVMFDLSETGINSIDMDFVRFIINCFKVYYPKYLSKIVIFDMPWLMNAAFKIVKTWLGPEAVSLLKFTSKNEVQDYVSVEYLPPHMGGTDPFKYSYPPLVDDDFQTPLCENGPITSEDETSSKEDIESDGKETLETISNEEQTPLLKKINPTESTSKAEENEKVDSKVKAFKKPLSVFKGPLLHISPAEELYFGSTESGEKKTLIVLTNVTKNIVAFKVRTTAPEKYRVKPSNSSCDPGASVDIVVSPHGGLTVSAQDRFLIMAAEMEQSSGTGPAELTQFWKEVPRNKVMEHRLRCHTVESSKPNTLTLKDNAFNMSDKTSEDICLQLSRLLESNRKLEDQVQRCIWFQQLLLSLTMLLLAFVTSFFYLLYS

SEQ ID NO: 2 - protein, 455 aa, Homo sapiens
  motile sperm domain containing 2, protein variant 2
MLDESFQWRKEISVNDLNESSIPRWLLEIGVIYLHGYDKEGNKLFWIRVKYHVKDQKTILDKKKLIAFWLERYAKRENGKPVTVMFDLSETGINSIDMDFVRFIINCFKVYYPKYLSKIVIFDMPWLMNAAFKIVKTWLGPEAVSLLKFTSKNEVQDYVSVEYLPPHMGGTDPFKYSYPPLVDDDFQTPLCENGPITSEDETSSKEDIESDGKETLETISNEEQTPLLKKINPTESTSKAEENEKVDSKVKAFKKPLSVFKGPLLHISPAEELYFGSTESGEKKTLIVLTNVTKNIVAFKVRTTAPEKYRVKPSNSSCDPGASVDIVVSPHGGLTVSAQDRFLIMAAEMEQSSGTGPAELTQFWKEVPRNKVMEHRLRCHTVESSKPNTLTLKDNAFNMSDKTSEDICLQLSRLLESNRKLEDQVQRCIWFQQLLLSLTMLLLAFVTSFFYLLYS

SEQ ID NO: 3 - protein, 486 aa, Homo sapiens
  motile sperm domain containing 2, protein variant X1
MAENHAQNKAKLISETRRRFEAEYVTDKSDKYDARDVERLQQDDNWVESYLSWRHNIVDETLKMLDESFQWRKEISVNDLNESSIPRWLLEIGVIYLHGYDKEGNKLFWIRVKYHVKDQKTILDKKKLIAFWLERYAKRENGKPVTVMFDLSETGINSIDMDFVRFIINCFKVYYPKYLSKIVIFDMPWLMNAAFKIVKTWLGPEAVSLLKFTSKNEVQDYVSVEYLPPHMGGTDPFKYSYPPLVDDDFQTPLCENGPITSEDETSSKEDIESDGKETLETISNEEQTPLLKKINPTESTSKAEENEKVDSKVKAFKKPLSVFKGPLLHISPAEELYFGSTESGEKKTLIVLTNVTKNIVAFKVRTTAPEKYRVKPSNSSCDPGASVDIVVSPHGGLTVSAQDRFLIMAAEMEQSSGTGPAELTQFWKEVPRNKVMEHRLRCHTVESSKPNTLTLKDNAFNMSDKTSEDICLQFATSSCEMDCSPP

SEQ ID NO: 4 - protein, 475 aa, Homo sapiens
  motile sperm domain containing 2, protein variant X2
MAENHAQNKAKLISETRRRFEAEYVTDKSDKYDARDVERLQQDDNWVESYLSWRHNIVDETLKMLDESFQWRKEISVNDLNESSIPRWLLEIGVIYLHGYDKEGNKLFWIRVKYHVKDQKTILDKKKLIAFWLERYAKRENGKPVTVMFDLSETGINSIDMDFVRFIINCFKVYYPKYLSKIVIFDMPWLMNAAFKIVKTWLGPEAVSLLKFTSKNEVQDYVSVEYLPPHMGGTDPFKYSYPPLVDDDFQTPLCENGPITSEDETSSKEDIESDGKETLETISNEEQTPLLKKINPTESTSKAEENEKVDSKVKAFKKPLSVFKGPLLHISPAEELYFGSTESGEKKTLIVLTNVTKNIVAFKVRTTAPEKYRVKPSNSSCDPGASVDIVVSPHGGLTVSAQDRFLIMAAEMEQSSGTGPAELTQFWKEVPRNKVMEHRLRCHTVESSKPNTLTLKDNAFNMSDKTSEDICLQYS

SEQ ID NO: 5 - DNA, 3219 bp, Homo sapiens
  motile sperm domain containing 2, transcript variant 1, mRNA, coding region 125-1678
accgcctccccctcccacccttctctgtctacctctgggcgggactgccgggtgatgagatactcggtcggcgacggtagaacgggcgacggcgacaaccgcaatcacatccacgacggtgatcatggcagagaatcacgcccagaataaagccaagctcatctctgagacccggaggaggttcgaagctgagtatgtgacagataagtcagataaatatgatgcacgtgatgttgaaaggctacaacaagatgataactgggttgaaagttacttatcttggagacataatattgtagatgaaacactgaagatgctcgatgagagttttcagtggaggaaagaaatttctgtcaatgaccttaatgaatcctccattcccagatggttattggaaattggtgttatttatctccatggttatgacaaagaaggtaacaaattgttctggatcagggtgaagtatcatgtaaaagaccagaaaaccatattggacaaaaagaagctcatagcattctggttggaacgttatgctaagagggaaaatgggaaacctgtaacagtgatgtttgacctgtcagaaactggaataaatagcattgacatggactttgtacgctttatcatcaactgctttaaggtttattaccctaaatacctctcaaaaatagtgatctttgatatgccttggttaatgaatgctgctttcaaaattgtgaaaacctggcttggtccagaagcagtgagcttgttgaagtttacaagcaaaaatgaagtccaggactatgtcagtgtagaatacctgcctccccacatgggtggaactgatcctttcaagtatagctatccaccactagtagatgatgacttccagaccccactgtgtgagaatgggcctattaccagtgaggatgaaacttcaagtaaagaagacatagaaagtgatggcaaagaaacattggaaacaatttctaatgaagaacaaacacctcttcttaaaaagattaacccaaccgaatctacttccaaagcagaagaaaatgaaaaagttgattcaaaagtgaaagctttcaagaaaccattgagtgtatttaaaggccccttactacacatcagcccagcagaagaactgtactttggaagtacagaatccggagagaagaaaaccttaatagtgttgacaaatgtaactaaaaatatagtggcatttaaggtgagaacaacagctccagaaaaatacagagtcaagccaagcaatagcagctgtgacccgggtgcatcagtggatatagttgtgtctccccatgggggtttaacagtctctgcccaagaccgttttctgataatggctgcagaaatggaacagtcatctggcacaggcccagcagaattaactcagttttggaaagaagttcccagaaacaaagtgatggaacataggttaagatgccatactgttgaaagcagtaaaccaaacactcttacgttaaaagacaatgctttcaatatgtcagataaaaccagtgaagatatatgtctacaactcagtcgtttactagaaagcaataggaagcttgaagaccaagttcagcgttgtatctggttccagcagctgctgctttccttaacaatgctcttgcttgcttttgtcacctctttcttctatttattgtacagttaaagaagtggtgccgggtaggaaccacggttccttcgtccattagttggaaaaagtaacagacctaaaactctaccaagctactaaaaacattgcacatctgtgcttcctaaaaggaaatatgcagcacgtggaggggaacacatacatgtcttgaaaataaactgctagaataaagaaatgctggagaaattgattataagagactatagctatttagtaaagtaagtaaaggcatatccattgtgtaaattaatagtttaaatataatttattttttccttttgatctgaatacttttaaagcttaagttttatcgtgtaaatacattagctaaactgaaaagtataagtaacatgctttgttgcagccaaaaaatgtaatctgcttttttatgacagaattattatagctgagctgacttactagcttttctatactatgtatatagaagaacatgtatattgagaaagaaaacatacttatatagaggaatttatgtaaccatgactttgtaattttgagaattcctcccagtgatggtcagtattcttttggaatgtaaaccgatttaatgccaaaccaccttaacctttgtttctcagtgttccttaacagcctgccttttattaatctcaggcttttttatgaacactctcatttcagtagaatttggaaaactaagcgtggttggaatttctttgaattctgttagtaatgcccaaaagaaaagtctcaagcagtccccctatccagtcatttttatggagtttcatgttgtccactatagctggacactgaaccttttgcctaatttattataaaggcctgaccctctattgtcccatcttcacccccattccagagcagaggagtctctgtggaccatgaattgcactgtctccctcctcatttctaaatgaaaggtattagatataaatttttttgaaaggttagttgtttgagatgctaagcaggataataaatttagattttaaaatgttccctgtaaaagtcagcccatgacaaggaaatttacaaaatactagagtatctagaagggtgaaaacaaaaaaaaataaaaagaaacacagacgcccaggtgtcagctctccgtttaaagaatgaaaaatgtaactcatgatgatctgtgaaaccttcaaactaggaccaattgacttacttgatattctgcctttgatatggtagtacccacccggtattcctaaaatcctaaaaagatacaccttgcagtagcagaggcaatgacatgagtttgttttctcattaatatgaccagtttgggtctatgttggttcacatgtacatctactttatatgaaagaaaaaacagttgtctgcctgtaaaatgttgagtttcgattgagccatgtttggagattttattactattctgaagggtagtgttgttggttttcatcttcaagaagttgattccaaaactgagttatgaagaatgatataacagttccttcaaaattggcctaggaaataaaaccttaaaaggacaaaaaaaaaaa

SEQ ID NO: 6 - DNA, 3183 bp, Homo sapiens
  motile sperm domain containing 2, transcript variant 2, mRNA, coding region 278-1642
agtcacaataataggtacttaaaaacatgtcatatgataggaaactagaataacacacctctaaataatccatggattaccaacttctcagcaatggtgtaaattcttctgctaaataacccgtgggttaaagaggacatcacattggaaattccagagtacttaaaataagtcagataaatatgatgcacgtgatgttgaaaggctacaacaagatgataactgggttgaaagttacttatcttggagacataatattgtagatgaaacactgaagatgctcgatgagagttttcagtggaggaaagaaatttctgtcaatgaccttaatgaatcctccattcccagatggttattggaaattggtgttatttatctccatggttatgacaaagaaggtaacaaattgttctggatcagggtgaagtatcatgtaaaagaccagaaaaccatattggacaaaaagaagctcatagcattctggttggaacgttatgctaagagggaaaatgggaaacctgtaacagtgatgtttgacctgtcagaaactggaataaatagcattgacatggactttgtacgctttatcatcaactgctttaaggtttattaccctaaatacctctcaaaaatagtgatctttgatatgccttggttaatgaatgctgctttcaaaattgtgaaaacctggcttggtccagaagcagtgagcttgttgaagtttacaagcaaaaatgaagtccaggactatgtcagtgtagaatacctgcctccccacatgggtggaactgatcctttcaagtatagctatccaccactagtagatgatgacttccagaccccactgtgtgagaatgggcctattaccagtgaggatgaaacttcaagtaaagaagacatagaaagtgatggcaaagaaacattggaaacaatttctaatgaagaacaaacacctcttcttaaaaagattaacccaaccgaatctacttccaaagcagaagaaaatgaaaaagttgattcaaaagtgaaagctttcaagaaaccattgagtgtatttaaaggccccttactacacatcagcccagcagaagaactgtactttggaagtacagaatccggagagaagaaaaccttaatagtgttgacaaatgtaactaaaaatatagtggcatttaaggtgagaacaacagctccagaaaaatacagagtcaagccaagcaatagcagctgtgacccgggtgcatcagtggatatagttgtgtctccccatgggggtttaacagtctctgcccaagaccgttttctgataatggctgcagaaatggaacagtcatctggcacaggcccagcagaattaactcagttttggaaagaagttcccagaaacaaagtgatggaacataggttaagatgccatactgttgaaagcagtaaaccaaacactcttacgttaaaagacaatgctttcaatatgtcagataaaaccagtgaagatatatgtctacaactcagtcgtttactagaaagcaataggaagcttgaagaccaagttcagcgttgtatctggttccagcagctgctgctttccttaacaatgctcttgcttgcttttgtcacctctttcttctatttattgtacagttaaagaagtggtgccgggtaggaaccacggttccttcgtccattagttggaaaaagtaacagacctaaaactctaccaagctactaaaaacattgcacatctgtgcttcctaaaaggaaatatgcagcacgtggaggggaacacatacatgtcttgaaaataaactgctagaataaagaaatgctggagaaattgattataagagactatagctatttagtaaagtaagtaaaggcatatccattgtgtaaattaatagtttaaatataatttattttttccttttgatctgaatacttttaaagcttaagttttatcgtgtaaatacattagctaaactgaaaagtataagtaacatgctttgttgcagccaaaaaatgtaatctgcttttttatgacagaattattatagctgagctgacttactagcttttctatactatgtatatagaagaacatgtatattgagaaagaaaacatacttatatagaggaatttatgtaaccatgactttgtaattttgagaattcctcccagtgatggtcagtattcttttggaatgtaaaccgatttaatgccaaaccaccttaacctttgtttctcagtgttccttaacagcctgccttttattaatctcaggcttttttatgaacactctcatttcagtagaatttggaaaactaagcgtggttggaatttctttgaattctgttagtaatgcccaaaagaaaagtctcaagcagtccccctatccagtcatttttatggagtttcatgttgtccactatagctggacactgaaccttttgcctaatttattataaaggcctgaccctctattgtcccatcttcacccccattccagagcagaggagtctctgtggaccatgaattgcactgtctccctcctcatttctaaatgaaaggtattagatataaatttttttgaaaggttagttgtttgagatgctaagcaggataataaatttagattttaaaatgttccctgtaaaagtcagcccatgacaaggaaatttacaaaatactagagtatctagaagggtgaaaacaaaaaaaaataaaaagaaacacagacgcccaggtgtcagctctccgtttaaagaatgaaaaatgtaactcatgatgatctgtgaaaccttcaaactaggaccaattgacttacttgatattctgcctttgatatggtagtacccacccggtattcctaaaatcctaaaaagatacaccttgcagtagcagaggcaatgacatgagtttgttttctcattaatatgaccagtttgggtctatgttggttcacatgtacatctactttatatgaaagaaaaaacagttgtctgcctgtaaaatgttgagtttcgattgagccatgtttggagattttattactattctgaagggtagtgttgttggttttcatcttcaagaagttgattccaaaactgagttatgaagaatgatataacagttccttcaaaattggcctaggaaataaaaccttaaaaggacaaaaaaaaaaa

SEQ ID NO: 7 - DNA, 2330 bp, Homo sapiens
  motile sperm domain containing 2, transcript variant X1, mRNA, coding region 125-1582
accgcctccccctcccacccttctctgtctacctctgggcgggactgccgggtgatgagatactcggtcggcgacggtagaacgggcgacggcgacaaccgcaatcacatccacgacggtgatcatggcagagaatcacgcccagaataaagccaagctcatctctgagacccggaggaggttcgaagctgagtatgtgacagataagtcagataaatatgatgcacgtgatgttgaaaggctacaacaagatgataactgggttgaaagttacttatcttggagacataatattgtagatgaaacactgaagatgctcgatgagagttttcagtggaggaaagaaatttctgtcaatgaccttaatgaatcctccattcccagatggttattggaaattggtgttatttatctccatggttatgacaaagaaggtaacaaattgttctggatcagggtgaagtatcatgtaaaagaccagaaaaccatattggacaaaaagaagctcatagcattctggttggaacgttatgctaagagggaaaatgggaaacctgtaacagtgatgtttgacctgtcagaaactggaataaatagcattgacatggactttgtacgctttatcatcaactgctttaaggtttattaccctaaatacctctcaaaaatagtgatctttgatatgccttggttaatgaatgctgctttcaaaattgtgaaaacctggcttggtccagaagcagtgagcttgttgaagtttacaagcaaaaatgaagtccaggactatgtcagtgtagaatacctgcctccccacatgggtggaactgatcctttcaagtatagctatccaccactagtagatgatgacttccagaccccactgtgtgagaatgggcctattaccagtgaggatgaaacttcaagtaaagaagacatagaaagtgatggcaaagaaacattggaaacaatttctaatgaagaacaaacacctcttcttaaaaagattaacccaaccgaatctacttccaaagcagaagaaaatgaaaaagttgattcaaaagtgaaagctttcaagaaaccattgagtgtatttaaaggccccttactacacatcagcccagcagaagaactgtactttggaagtacagaatccggagagaagaaaaccttaatagtgttgacaaatgtaactaaaaatatagtggcatttaaggtgagaacaacagctccagaaaaatacagagtcaagccaagcaatagcagctgtgacccgggtgcatcagtggatatagttgtgtctccccatgggggtttaacagtctctgcccaagaccgttttctgataatggctgcagaaatggaacagtcatctggcacaggcccagcagaattaactcagttttggaaagaagttcccagaaacaaagtgatggaacataggttaagatgccatactgttgaaagcagtaaaccaaacactcttacgttaaaagacaatgctttcaatatgtcagataaaaccagtgaagatatatgtctacaatttgccacctccagctgtgaaatggactgcagtccaccctaagtactgtgcacagtatctccctgtgtgtgtgcacagtggcttccccttacatggtagatttttggccttaatataatctaatcccaaagtagttgtgtatgttttctgttccttggcaaataaatgaagaaataattagccaagattgaaaatgtattgtcctaacggtgtccctttaatgtttcatatgaaaaattatgttgacccactaaaatatccttgctcaatgtctggtcagttgaatttaataacatatcttgttaatgtttgtgtgtctattaaatgtgactaagcaggattactgaaaattcactataaaatcaaaggcatctaaacgtttgtacttgtcttgattaatcatatatttacacttgatttttttctgtcttcatttgtttttatttaatcataattgcatgatttttttggtactctaatcagtaattttatttttaatcatgtcattacctattcatgaccaaattaccaaggaaccaacatttagatttagatatttgttttcacttaggaatggaaattaatagattttccatgaaagcattagtgaaatatcattaccttgatctgcaagtagcctaaaaatgcgattgctggtaaacctggcctcaaatttcatactaccataactgtttttatatattgccactaattttgactggatttaatagcactttattgtacaactacaaaaaaaaatatattcctagaattgttgccagtgtaa

SEQ ID NO: 8 - DNA, 3909 bp, Homo sapiens
  motile sperm domain containing 2, transcript variant X2, mRNA, coding region 125-1549
accgcctccccctcccacccttctctgtctacctctgggcgggactgccgggtgatgagatactcggtcggcgacggtagaacgggcgacggcgacaaccgcaatcacatccacgacggtgatcatggcagagaatcacgcccagaataaagccaagctcatctctgagacccggaggaggttcgaagctgagtatgtgacagataagtcagataaatatgatgcacgtgatgttgaaaggctacaacaagatgataactgggttgaaagttacttatcttggagacataatattgtagatgaaacactgaagatgctcgatgagagttttcagtggaggaaagaaatttctgtcaatgaccttaatgaatcctccattcccagatggttattggaaattggtgttatttatctccatggttatgacaaagaaggtaacaaattgttctggatcagggtgaagtatcatgtaaaagaccagaaaaccatattggacaaaaagaagctcatagcattctggttggaacgttatgctaagagggaaaatgggaaacctgtaacagtgatgtttgacctgtcagaaactggaataaatagcattgacatggactttgtacgctttatcatcaactgctttaaggtttattaccctaaatacctctcaaaaatagtgatctttgatatgccttggttaatgaatgctgctttcaaaattgtgaaaacctggcttggtccagaagcagtgagcttgttgaagtttacaagcaaaaatgaagtccaggactatgtcagtgtagaatacctgcctccccacatgggtggaactgatcctttcaagtatagctatccaccactagtagatgatgacttccagaccccactgtgtgagaatgggcctattaccagtgaggatgaaacttcaagtaaagaagacatagaaagtgatggcaaagaaacattggaaacaatttctaatgaagaacaaacacctcttcttaaaaagattaacccaaccgaatctacttccaaagcagaagaaaatgaaaaagttgattcaaaagtgaaagctttcaagaaaccattgagtgtatttaaaggccccttactacacatcagcccagcagaagaactgtactttggaagtacagaatccggagagaagaaaaccttaatagtgttgacaaatgtaactaaaaatatagtggcatttaaggtgagaacaacagctccagaaaaatacagagtcaagccaagcaatagcagctgtgacccgggtgcatcagtggatatagttgtgtctccccatgggggtttaacagtctctgcccaagaccgttttctgataatggctgcagaaatggaacagtcatctggcacaggcccagcagaattaactcagttttggaaagaagttcccagaaacaaagtgatggaacataggttaagatgccatactgttgaaagcagtaaaccaaacactcttacgttaaaagacaatgctttcaatatgtcagataaaaccagtgaagatatatgtctacaatacagttaaagaagtggtgccgggtaggaaccacggttccttcgtccattagttggaaaaagtaacagacctaaaactctaccaagctactaaaaacattgcacatctgtgcttcctaaaaggaaatatgcagcacgtggaggggaacacatacatgtcttgaaaataaactgctagaataaagaaatgctggagaaattgattataagagactatagctatttagtaaagtaagtaaaggcatatccattgtgtaaattaatagtttaaatataatttattttttccttttgatctgaatacttttaaagcttaagttttatcgtgtaaatacattagctaaactgaaaagtataagtaacatgctttgttgcagccaaaaaatgtaatctgcttttttatgacagaattattatagctgagctgacttactagcttttctatactatgtatatagaagaacatgtatattgagaaagaaaacatacttatatagaggaatttatgtaaccatgactttgtaattttgagaattcctcccagtgatggtcagtattcttttggaatgtaaaccgatttaatgccaaaccaccttaacctttgtttctcagtgttccttaacagcctgccttttattaatctcaggcttttttatgaacactctcatttcagtagaatttggaaaactaagcgtggttggaatttctttgaattctgttagtaatgcccaaaagaaaagtctcaagcagtccccctatccagtcatttttatggagtttcatgttgtccactatagctggacactgaaccttttgcctaatttattataaaggcctgaccctctattgtcccatcttcacccccattccagagcagaggagtctctgtggaccatgaattgcactgtctccctcctcatttctaaatgaaaggtattagatataaatttttttgaaaggttagttgtttgagatgctaagcaggataataaatttagattttaaaatgttccctgtaaaagtcagcccatgacaaggaaatttacaaaatactagagtatctagaagggtgaaaacaaaaaaaaataaaaagaaacacagacgcccaggtgtcagctctccgtttaaagaatgaaaaatgtaactcatgatgatctgtgaaaccttcaaactaggaccaattgacttacttgatattctgcctttgatatggtagtacccacccggtattcctaaaatcctaaaaagatacaccttgcagtagcagaggcaatgacatgagtttgttttctcattaatatgaccagtttgggtctatgttggttcacatgtacatctactttatatgaaagaaaaaacagttgtctgcctgtaaaatgttgagtttcgattgagccatgtttggagattttattactattctgaagggtagtgttgttggttttcatcttcaagaagttgattccaaaactgagttatgaagaatgatataacagttccttcaaaattggcctaggaaataaaaccttaaaaggacactggtgtgctactttgtcttaatttgggcttttctgtttcagtttgccacctccagctgtgaaatggactgcagtccaccctaagtactgtgcacagtatctccctgtgtgtgtgcacagtggcttccccttacatggtagatttttggccttaatataatctaatcccaaagtagttgtgtatgttttctgttccttggcaaataaatgaagaaataattagccaagattgaaaatgtattgtcctaacggtgtccctttaatgtttcatatgaaaaattatgttgacccactaaaatatccttgctcaatgtctggtcagttgaatttaataacatatcttgttaatgtttgtgtgtctattaaatgtgactaagcaggattactgaaaattcactataaaatcaaaggcatctaaacgtttgtacttgtcttgattaatcatatatttacacttgatttttttctgtcttcatttgtttttatttaatcataattgcatgatttttttggtactctaatcagtaattttatttttaatcatgtcattacctattcatgaccaaattaccaaggaaccaacatttagatttagatatttgttttcacttaggaatggaaattaatagattttccatgaaagcattagtgaaatatcattaccttgatctgcaagtagcctaaaaatgcgattgctggtaaacctggcctcaaatttcatactaccataactgtttttatatattgccactaattttgactggatttaatagcactttattgtacaactacaaaaaaaaatatattcctagaattgttgccagtgtaa

SEQ ID NO: 9 - DNA, 58 bp, Artificial Sequence
  shRNA hairpin sequence #1 for MOSPD2
ccggcccagatggttattggaaattctcgagatttccaataaccatctgggttttttg

SEQ ID NO: 10 - DNA, 21 bp, Artificial Sequence
  target sequence on MOSPD2 for shRNA hairpin sequence #1
cccagatggttattggaaatt

SEQ ID NO: 11 - DNA, 59 bp, Artificial Sequence
  shRNA hairpin sequence #2 for MOSPD2
ccgggccatactgttgaaagcagtactcgagtactgctttcaacagtatggcttttttg

SEQ ID NO: 12 - DNA, 21 bp, Artificial Sequence
  MOSPD2 target sequence for shRNA hairpin sequence #2
gccatactgttgaaagcagta

SEQ ID NO: 13 - DNA, 59 bp, Artificial Sequence
  shRNA hairpin sequence #3 for MOSPD2
ccggccctcctcatttctaaatgaactcgagttcatttagaaatgaggagggttttttg

SEQ ID NO: 14 - DNA, 21 bp, Artificial Sequence
  MOSPD2 target sequence for shRNA hairpin sequence #3
ccctcctcatttctaaatgaa

SEQ ID NO: 15 - protein, 9 aa, Artificial Sequence
  Hemagglutinin tag for MOSPD2
YPYDVPDYA